European Patent Application EP 4 407 023 A1, published July 31, 2024. Title: 一种延长寿命、抗衰老、减脂的罗伊氏乳杆菌及其产品与应用. Applicant: 广西爱生生命科技有限公司. Application CN. The sequence listing filed with the application follows.

SEQUENCE LISTING (29 sequences)

SEQ ID NO: 1 - DNA, 20 bp, synthetic construct
  source 1..20: mol_type = other DNA
gcttcactcgctgcagttaa

SEQ ID NO: 2 - DNA, 20 bp, synthetic construct
  source 1..20: mol_type = other DNA
ccaaccaaacctcggtcaga

SEQ ID NO: 3 - DNA, 20 bp, synthetic construct
  source 1..20: mol_type = other DNA
agagtttgatcctggctcag

SEQ ID NO: 4 - DNA, 22 bp, synthetic construct
  source 1..22: mol_type = other DNA
tacggctaccttgttacgactt

SEQ ID NO: 5 - DNA, 1485 bp, Lactobacillus reuteri
  source 1..1485: mol_type = genomic DNA
gagggacgggcgggtgctatacatgcaagtcgtacgcactggcccaactgattgatggtgcttgcacctgattgacgatggatcaccagtgagtggcggacgggtgagtaacacgtaggtaacctgccccggagcgggggataacatttggaaacagatgctaataccgcataacaacaaaagccgcatggcttttgtttgaaagatggctttggctatcactctgggatggacctgcggtgcattagctagttggtaaggtaacggcttaccaaggcgatgatgcatagccgagttgagagactgatcggccacaatggaactgagacacggtccatactcctacgggaggcagcagtagggaatcttccacaatgggcgcaagcctgatggagcaacaccgcgtgagtgaagaagggtttcggctcgtaaagctctgttgttggagaagaacgtgcgtgagagtaactgttcacgcagtgacggtatccaaccagaaagtcacggctaactacgtgccagcagccgcggtaatacgtaggtggcaagcgttatccggatttattgggcgtaaagcgagcgcaggcggttgcttaggtctgatgtgaaagccttcggcttaaccgaagaagtgcatcggaaaccgggcgacttgagtgcagaagaggacagtggaactccatgtgtagcggtggaatgcgtagatatatggaagaacaccagtggcgaagggcggctgtctggtctgcaactgacgctgaggctcgaaagcatgggtagcgaacaggattagataccctggtagtccatgccgtaaacgatgagtgctaggtgttggagggtttccgcccttcagtgccggagctaacgcattaagcactccgcctggggagtacgaccgcaaggttgaaactcaaaggaattgacgggggcccgcacaagcggtggagcatgtggtttaattcgaagctacgcgaagaaccttaccaggtcttgacatcttgcgctaaccttagagataaggcgttcccttcggggacgcaatgacaggtggtgcatggtcgtcgtcagctcgtgtcgtgagatgttgggttaagtcccgcaacgagcgcaacccttgttactagttgccagcattgagttgggcactctagtgagactgccggtgacaaaccggaggaaggtggggacgacgtcagatcatcatgccccttatgacctgggctacacacgtgctacaatggacggtacaacgagtcgcaaactcgcgagagtaagctaatctcttaaagccgttctcagttcggactgtaggctgcaactcgcctacacgaagtcggaatcgctagtaatcgcggatcagcatgccgcggtgaatacgttcccgggccttgtacacaccgcccgtcacaccatgggagtttgtaacgcccaaagtcggtggcctaacctttatggaggggaccgcgcccccccctataacgc

SEQ ID NO: 6 - DNA, 23 bp, synthetic construct
  source 1..23: mol_type = other DNA
ctacgaacttcctgacggacaag

SEQ ID NO: 7 - DNA, 17 bp, synthetic construct
  source 1..17: mol_type = other DNA
ccggcggactccatacc

SEQ ID NO: 8 - DNA, 23 bp, synthetic construct
  source 1..23: mol_type = other DNA
ctaacttcaagccaatgccacta

SEQ ID NO: 9 - DNA, 23 bp, synthetic construct
  source 1..23: mol_type = other DNA
tccagcttgactcagctcatgtc

SEQ ID NO: 10 - DNA, 20 bp, synthetic construct
  source 1..20: mol_type = other DNA
ctccaagcacactctcccag

SEQ ID NO: 11 - DNA, 20 bp, synthetic construct
  source 1..20: mol_type = other DNA
tccctttcgaaacagcctcg

SEQ ID NO: 12 - DNA, 22 bp, synthetic construct
  source 1..22: mol_type = other DNA
tttgcattttctcgtctctgtc

SEQ ID NO: 13 - DNA, 21 bp, synthetic construct
  source 1..21: mol_type = other DNA
tctatttccagcacacctcgt

SEQ ID NO: 14 - DNA, 21 bp, synthetic construct
  source 1..21: mol_type = other DNA
ggtgcagttgcttcgaatctt

SEQ ID NO: 15 - DNA, 22 bp, synthetic construct
  source 1..22: mol_type = other DNA
tcttccttgaaccgcttctttc

SEQ ID NO: 16 - DNA, 22 bp, synthetic construct
  source 1..22: mol_type = other DNA
aattccgatttccagcttcttc

SEQ ID NO: 17 - DNA, 25 bp, synthetic construct
  source 1..25: mol_type = other DNA
tctgcagatttggtgcatactataa

SEQ ID NO: 18 - DNA, 22 bp, synthetic construct
  source 1..22: mol_type = other DNA
ggcaaaccgtgattttcacatt

SEQ ID NO: 19 - DNA, 20 bp, synthetic construct
  source 1..20: mol_type = other DNA
tcacgagcccattcgatgac

SEQ ID NO: 20 - DNA, 24 bp, synthetic construct
  source 1..24: mol_type = other DNA
tccaatgccagctgaaacaacacc

SEQ ID NO: 21 - DNA, 24 bp, synthetic construct
  source 1..24: mol_type = other DNA
tggaatggctgacacggttgaatg

SEQ ID NO: 22 - DNA, 20 bp, synthetic construct
  source 1..20: mol_type = other DNA
cgcattcgccaagagaaacc

SEQ ID NO: 23 - DNA, 22 bp, synthetic construct
  source 1..22: mol_type = other DNA
acgttgacattgtctcggatga

SEQ ID NO: 24 - DNA, 21 bp, synthetic construct
  source 1..21: mol_type = other DNA
tacagaacgtccaaccacatc

SEQ ID NO: 25 - DNA, 21 bp, synthetic construct
  source 1..21: mol_type = other DNA
gcccttctctccagcaatatc

SEQ ID NO: 26 - DNA, 23 bp, synthetic construct
  source 1..23: mol_type = other DNA
gagcttcggagttgttctctatg

SEQ ID NO: 27 - DNA, 22 bp, synthetic construct
  source 1..22: mol_type = other DNA
cttccgggccattccaatataa

SEQ ID NO: 28 - DNA, 22 bp, synthetic construct
  source 1..22: mol_type = other DNA
gtgacgagcttcgatcgattag

SEQ ID NO: 29 - DNA, 21 bp, synthetic construct
  source 1..21: mol_type = other DNA
ggacgatggctttgtcgatta